European Patent Specification EP 3 189 150 B1, published March 18, 2026. Title: METHOD AND MICROORGANISM FOR PRODUCTION OF METHIONINE BY FERMENTATION WITH IMPROVED METHIONINE EFFLUX. Applicant: METABOLIC EXPLORER. The sequence listing filed with the application follows.

SEQUENCE LISTING (37 sequences)

SEQ ID NO: 1 - protein, 245 aa, Escherichia coli
MESPTPQPAPGSATFMEGCKDSLPIVISYIPVAFAFGLNATRLGFSPLESVFFSCIIYAGASQFVITAMLAAGSSLWIAALTVMAMDVRHVLYGPSLRSRIIQRLQKSKTALWAFGLTDEVFAAATAKLVRNNRRWSENWMIGIAFSSWSSWVFGTVIGAFSGSGLLQGYPAVEAALGFMLPALFMSFLLASFQRKQSLCVTAALVGALAGVTLFSIPVAILAGIVCGCLTALIQAFWQGAPDEL

SEQ ID NO: 2 - protein, 111 aa, Escherichia coli
MSYEVLLLGLLVGVANYCFRYLPLRLRVGNARPTKRGAVGILLDTIGIASICALLVVSTAPEVMHDTRRFVPTLVGFAVLGASFYKTRSIIIPTLLSALAYGLAWKVMAII

SEQ ID NO: 3 - protein, 244 aa, Citrobacter koseri
MESPAPQSEPRPATLTEGFKDSLPIVISYIPVAFAFGLNATRLGFTPLESVFFSCIIYAGASQFVITTMLAAGSTLWVAALTVMAMDVRHVLYGPSLRSRISQRLSKPKTALWAFGLTDEVFAAATAKLVRDNRRWSEWMIGIAFCSWASWVLGTVIGAFSGSGLLKGFPAVEAALGFMLPALFMSFLLASFQRKQTLCVTAALIGALAGVTLFSIPAAILAGIASGCLTALIQSFWQGAPDEL

SEQ ID NO: 4 - protein, 111 aa, Citrobacter koseri
MSYEVLLLGLLVGCANYCFRYLPLRLRMGNTRPARRGATGVLLDTIGIASICALLVVSTAPEVMHDASRFIPTLVGFAVLGVSFYKTRSIIIPTLLSALGYGLAWKIEVIL

SEQ ID NO: 5 - protein, 245 aa, Shigella flexneri
MESPVPQSESRSATLTEGFKDSLPIVISYIPVAFAFGMNATRLGFTPVESVFFSCIIYAGASQFVITTMLAAGSSLWVAALTVMAMDVRHVLYGPSLRSRIARQLSKPKSALWAFGLTDEVFAAATAKLVRDNRRWSENWMIGIALCSWASWVLGTVIGAFSGTGLLKGFPAVEAALGFMLPALFMSFLLASFQRNQTLCVTAALAGALAGVTLFSIPAAILAGIVCGCLTALIQSFWQGGPDEL

SEQ ID NO: 6 - protein, 111 aa, Shigella flexneri
MSYEVLLLGLLVGCVNYCFRYLPLRLRMGNVRPTKRGATGILLDTIGIASICALLVVSTAPEVMHDARRFVPTLVGFVVLGASFYKTRSIIIPTLLSALGYGLAWKMLFVL

SEQ ID NO: 7 - protein, 242 aa, Raoultella ornithinolytica
MEKPAPASEATLPEGIKDSLPIVISYIPVAFAFGLNATRLGFTPLESLFFSCIIYAGASQFVITAMLAAGSSLWVAALTVMAMDVRHVLYGPSLRSRIHRALDKRKTALWAFGLTDEVFAAATAKLVRDNRRWSESWMLGIAFTSWISWVFGTLIGAYSGSGLLVGFPAVEAALSFMLPALFMSFLLASFQRKQSLSVTAALAGALGGIILFSIPAAILAGIVCGCLAALIQASIQGMPDEQ

SEQ ID NO: 8 - protein, 113 aa, Raoultella ornithinolytica
MNNNVLIIGIVVGCVNYLFRYLPLRLRAGNARPTRRGPLSVLLDTIGIASICALLIVSSVPEILSDSRRLLPTLVGFTVLGLAFWKTRSIIMPTLLSALAYGIAWKITTFLYF

SEQ ID NO: 9 - protein, 250 aa, Enterobacter sp. (R4-368)
MDMDSSVTATKSTSDQSATFLEGIKDSLPIVLSYVPVAFAFGMNATKLGFTPLESVFFSCIIYAGASQFVITTMLAAGSALWVAALTVMAMDVRHVLYGPSLRSRILQPLKNRKTAVWAFGLTDEVFAAATAKLVRDNRRWSENWMIGIALFSWLSWVAGTVLGAFSGDGLLDGYPAVESALGFMLPALFMSFLLASFQRRQISAVTAALLGALAGVTLFSIPAAILAGIFAGCLAALVQAFYQGASDAQ

SEQ ID NO: 10 - protein, 111 aa, Enterobacter sp. (R4-368)
MRNEVLLLGLLVGCVNFLFRYLPLRIRAGQSRPAKRGVSGVFLDTIGIASICALLVVSCVPEIAADSRRLLPTLAGFAVLGVSFWKTRSIILPTLLSAFAYGIVWKLLADA

SEQ ID NO: 11 - protein, 257 aa, Yersinia enterocolitica subsp. Enterocolitica
MQSQTTDSPSTAQPTATFIEGITDSLPIVIGYLPVAFAFGLSSVKLGFTPWEAIFFSCIIYAGASQFVITALLSAGMSLWVSALTVMAMDVRHILYGPALKHRIVTRLSGKKTALWAFGLTDEVFAAATTKLMKDQRRWSENWMLGIAFTSWLSWVAGTAIGAMFGHGPLENYPAIEASLSFMLPALFLSFLLASFKRQYSLTVIASLTGALLGVLLFSIPVAILAGIGGGCLAALLQPVPETVIENNESDKEEPKP

SEQ ID NO: 12 - protein, 257 aa, Yersinia enterocolitica subsp. Enterocolitica; identical to SEQ ID NO: 11

SEQ ID NO: 13 - protein, 113 aa, Yersinia enterocolitica subsp. Enterocolitica
MNMDVVIIGLVVGTVNYLFRYLPLRLGPARKQAGLQRGKVSLLLDSIGIASICALLVVSSTPEIVHTPQKLIPTLIGFLVICGCFYKTNSIIFATLLGALSYGLTFKLLMILA

SEQ ID NO: 14 - protein, 113 aa, Yersinia enterocolitica subsp. Enterocolitica
MNMDVVIIGLVVGTVNYLFRYLPLRLGPARKQAGLQRGKVSLLLDSIGIASICALLVVSSTPEIVHNPQKLIPTLIGFLVICGCFYKTNSIIFATLLGALSYGLTFKLLMILA

SEQ ID NO: 15 - protein, 252 aa, Photorhabdus luminescens subsp. laumondii
MPVSDTSSPLTSKKSSFTEGIIDSLPIVIGYIPVAFAFGLNAVKLGFNPMEAIFFSCIIYAGASQFVITALLSAGTSLWISALTIMAMDVRHILYGPSLRHRIKDKLTEKKTVIWAFGLTDEVFAAATAKLIKNHRSWSENWMVAIAICSWLAWGAGTAAGAFLGNGYLESYPAIEAAMIFMLPALFLSFLLASCRKQNSYCVATALTGALLGITFFSIPVAILAGIVGGCIAALLQPQNNCNDSSEQKETP

SEQ ID NO: 16 - protein, 112 aa, Photorhabdus luminescens subsp.laumondii
MIDSKILLIGLFVGLANFSFRYLPLRFGKARQSAGRKAGKTSIILDSIGIASICSLLIVSGVPDVMRESQKLLPTLIGCLTICLVFYKTKQIILATLFGALLFGLTFKIFMN

SEQ ID NO: 17 - protein, 245 aa, Citrobacter youngae
MDSPIPQSGSRSATLTEGFKDSLPIVISYIPVAFAFGLNATRLGFTPVESVFLSCIIYAGASQFVITTMLAAGSSLWVAALTVMAMDVRHVLYGPSLRSRIAQRLSKPKSALWAFGLTDEVFAAATAKLVRDNRRWSENWMIGIALCSWASWVFGTAIGAFSGSGLLKDYPAVEAALGFMLPALFMSFLLASFQRKQALCVTVALTGALAGVILFSIPAAILLGIVCGCLTALLQSFWQGGPDEL

SEQ ID NO: 18 - protein, 111 aa, Citrobacter youngae
MSYEVLLLGLLVGCVNYCFRYLPLRLGAGNVRPARRGATGILLDTIGIASICALLVVSTAPEVMHDARRFVPTLVGFVILGASFYKTRSIIIPTLLSALGYGLAWKMLVGL

SEQ ID NO: 19 - protein, 245 aa, Citrobacter freundii
MESPVPQSESSSATLTEGFKDSLPIVISYIPVAFAFGLNATRLGFTPVESVFFSCIIYAGASQFVITTMLAAGSSLWVAALTVMAMDVRHVLYGPSLRSRIAQRLSKPKSALWAFGLTDEVFAAATAKLVRDNRRWSENWMIGIALCSWASWVFGTVLGAFSGSGLLKDYPAVEAALGFMLPALFMSFLLASFQRKQALCVTAALAGALAGVMLFSIPAAILAGIVCGCLTALIQSFWQGGPDEL

SEQ ID NO: 20 - protein, 111 aa, Citrobacter freundii
MSYEVLLLGLLVGCVNYCFRYLPLRLGVGNVRPTKRGATGILLDTIGITSICALLVVSTAPEVMHDARRFVPTLVGFVILGASFYKTRSIIIPTLLSALGYGLAWKMLVVL

SEQ ID NO: 21 - DNA, 100 bp, artificial
  Oligonucleotide YbeM
aacactgcaaaatcctgctatttgatttgtatgagtgataagtgtaacgccgaataatcgtcgttggcgaattttacgactctgacaggaggtggcaatg

SEQ ID NO: 22 - DNA, 100 bp, artificial
  Oligonucleotide YbeM
gagaaagtaaacgtaacatgatgacgacaattctgacgattcatgttccttcaacgccggggcgcgcatggaatatgctggtggcacttcaggcaggaaa

SEQ ID NO: 23 - DNA, 100 bp, artificial
  Oligonucleotide YpjC
tgaggaatagacaatgttagttagtaaaagcaacggatttaacgctagcgcagttttgggtagtggaagttataatgaaaataaatcttctaaacacatg

SEQ ID NO: 24 - DNA, 100 bp, artificial
  Oligonucleotide YpjC
tgcgctaaaagaaatgaatagaaccttttcgataatataagaaaaagtgattttcatgttggtttacttaagccaagtagtacgcgtagtgttattttag

SEQ ID NO: 25 - DNA, 45 bp, artificial
  Oligonucleotide FldA
aaattattcttgtatctttgttataatatgggaaagtgcaaccat

SEQ ID NO: 26 - DNA, 100 bp, artificial
  Oligonucleotide YtfA
cgttaatcagcaggttagccagccacaaaaagccattgagaaaattattgattttacatgggattattatattgctaatccttggtttttaaaaattgtg

SEQ ID NO: 27 - DNA, 100 bp, artificial
  Oligonucleotide YtfA
tcatctaccgcgcacgaataaaactgccatccggctggcgggtgaacaggacctgttgattattccccgtatcaatggttaagcccgtcaccacgccgct

SEQ ID NO: 28 - DNA, 50 bp, artificial
  Oligonucleotide YjbB
ttgagcgctggctggcaccgaatctggggtatgacgcggactgattcaca

SEQ ID NO: 29 - DNA, 50 bp, artificial
  Oligonucleotide YjbB
aatctgtcacttttccttacaacaaacagggcgctcaatgagtgccctgt

SEQ ID NO: 30 - DNA, 1063 bp, Citrobacter koseri
atggaaagccctgcaccccagtctgagccccgtccggcaacattaacggaaggattcaaagacagtttaccgatagtcataagttatattccggtggcgtttgcgtttggccttaacgccacccgtctgggctttactcccctcgaaagcgtttttttctcctgcattatttacgcaggcgccagccagttcgtcatcaccaccatgctcgcggcgggcagcacattatgggtcgccgcgctgaccgtgatggcgatggacgtgcgtcatgtgctgtacggcccttccctgcgtagtcgcatcagccaacggctcagtaaacctaaaaccgccctgtgggcatttggcctcaccgatgaagtgtttgctgccgccacggccaaactggtgcgggataaccgccgctggagtgaaaactggatgatcggcatcgcgttctgctcctgggcctcctgggtgctcggcacggtcattggcgcattttccgggagcggattgctgaaaggcttccccgccgttgaggcggcattaggttttatgctgccagccctgtttatgagctttttgctcgcttcttttcaacgcaaacaaacgctgtgcgtcacggcggcgttaatcggcgcgctggcaggcgtcacgctgttttccattcctgcggctatcctggcgggtatcgccagcgggtgtctgaccgccttgatccagtcgttctggcaaggagcgcccgatgagttatgaggttctgctgctgggactgctggtcggctgcgccaattattgttttcgttatttaccgcttcgtctgcgaatgggaaacacccgccccgccaggcgcggcgcaacgggcgtgttgctcgacaccattggcatcgcgtccatctgcgccctgctggtggtgtctacggctcccgaagtgatgcacgacgccagccggttcattccgacgctggtcgggtttgccgtcctgggcgtcagtttctacaagacgcgcagcatcatcatcccaacgctactgagcgctctgggctatggactcgcctggaagatagaggtcattttataa

SEQ ID NO: 31 - DNA, 1063 bp, Shigella flexneri
atggaaagccctgttccccagtctgaatcccgttctgcaacgttaactgaaggattcaaagacagcctaccgatagttatcagttatattccggtcgcatttgcatttggtatgaatgcgactcgcctgggctttactcccgttgaaagcgtttttttctcctgcatcatttacgctggcgccagccagtttgtcatcacaaccatgctcgccgcaggcagctcactgtgggtcgcggctctgaccgtcatggcgatggatgttcgccatgttttgtacggcccttctctgcgcagccgtatcgcccgacagctgagcaaacctaaaagcgcgctatgggcctttggcctcaccgacgaagtctttgccgcggcaacggccaagctggtgcgggataaccggcgctggagtgaaaactggatgatcggcatcgcgctatgctcctgggcttcctgggtacttggtacggttatcggcgcattttccggcactggcttactgaagggattcccggcggtagaagcggcgctggggtttatgctcccggcgctgtttatgagttttctgctggcctctttccagcgtaatcaaacgctatgcgtcacggcggctttagccggtgcgctggctggcgtgacgctgttttctatcccggcagccatcctcgcaggcatagtctgcggatgcctgaccgcgctcattcagtcgttctggcagggaggtcctgatgagttatgaggttctgctgctcggcctgctggtcggctgcgtcaattactgttttcgctatttaccactgcgtctgcgaatggggaatgtgcgcccgacaaaacgcggagccactggaatactactcgacaccatcggtattgcatcaatttgcgccctgctagtggtgtctactgcgccagaagtgatgcacgatgcccgtcgttttgtgcctacgctggtggggtttgtggtactgggtgcaagcttctataagacccgcagcatcatcattccgaccttactgagtgccctgggctatggattagcctggaaaatgctgtttgtcttatag

SEQ ID NO: 32 - DNA, 1060 bp, Raoultella ornithinolytica
atggaaaaaccggcaccggcaagcgaagcaaccctgccggaaggtattaaagatagcctgccgattgtgattagctatattccggttgcatttgcctttggtctgaatgcaacccgtctgggttttacaccgctggaaagcctgttttttagctgtattatctatgccggtgcaagccagtttgttattaccgcaatgctggcagcaggtagcagcctgtgggttgcagcactgaccgttatggcaatggatgttcgtcatgttctgtatggtccgagcctgcgtagccgtattcatcgtgcactggataaacgtaaaaccgcactgtgggcatttggcctgaccgatgaagtttttgcagcagcaaccgcaaaactggttcgtgataatcgtcgttggagcgaaagctggatgctgggtattgcatttaccagctggattagctgggtttttggcaccctgattggtgcatatagcggtagcggtctgctggttggttttccggcagttgaagcagccctgagctttatgctgcctgcactgtttatgagttttctgctggcaagctttcagcgtaaacagagcctgagcgttaccgcagcactggcaggcgcactgggtggtattattctgtttagcattccggcagcaattctggcaggtattgtttgtggttgtctggcagcgctgattcaggcaagcattcagggtatgccggatgaacaataacgttctgattattggtattgtggtgggctgtgtgaattacctgtttcgttatctgccgctgcgtctgcgtgcaggtaatgcacgtccgacccgtcgtggtccgctgagcgttctgctggataccattggcattgcaagcatttgtgcactgctgattgttagcagcgttccggaaattctgagcgatagccgtcgtctgctgccgaccctggttggttttaccgttctgggtctggcattttggaaaacccgtagcattattatgccgacactgctgagcgcactggcctatggtattgcatggaaaattaccacctttctgtatttttga

SEQ ID NO: 33 - DNA, 1078 bp, Enterobacter sp. (R4-368)
atggatatggatagcagcgttaccgcaaccaaaagcaccagcgatcagagcgcaacctttctggaaggtattaaagatagcctgccgattgttctgagctatgttccggttgcatttgcctttggtatgaatgcaaccaaactgggttttacaccgctggaaagcgtgttttttagctgtattatctatgccggtgcaagccagtttgttattaccaccatgctggcagcaggtagcgcactgtgggttgcagcactgaccgttatggcaatggatgttcgtcatgttctgtatggtccgagcctgcgtagccgtattctgcagccgctgaaaaatcgtaaaaccgcagtgtgggcatttggtctgaccgatgaagtttttgcagcagcaaccgcaaaactggttcgtgataatcgtcgttggagcgaaaattggatgattggtattgcactgtttagctggctgagctgggttgccggtacagttctgggtgcatttagcggtgatggtctgctggatggttatccggcagttgaaagtgcactgggctttatgctgcctgccctgtttatgagctttctgctggcaagctttcagcgtcgtcagattagcgcagttaccgcagcactgctgggtgcactggcaggcgttaccctgtttagcattccggcagcaattctggcaggcatttttgcaggttgtctggcagcactggttcaggccttttatcagggtgcaagtgatgcgcaatgaggttctgctgctgggcctgctggttggttgtgttaattttctgtttcgttatctgccgctgcgtattcgtgcaggtcagagccgtccggcaaaacgtggtgttagcggtgtttttctggataccattggcattgcaagcatttgtgccctgctggtagttagctgtgttccggaaattgcagcagatagccgtcgtctgctgccgaccctggcaggttttgcagtgctgggtgttagcttttggaaaacccgtagcattattctgccgacactgctgagcgcatttgcgtatggtattgtttggaaactgctggcagatgcctaa

SEQ ID NO: 34 - DNA, 1112 bp, Yersinia enterocolitica subsp. enterocolitica
atgcaaagccaaaccaccgactccccctcgacggcccagccgaccgccacctttattgaaggaataaccgatagcctaccgattgttatcggttatctacccgttgcttttgcctttggtttgagttcggtaaaacttggctttactccgtgggaagctattttcttttcttgcattatttatgccggagccagccaattcgttattaccgccctgctcagcgcggggatgtcattgtgggtttccgccttgaccgtgatggctatggatgtccgccatatcttgtacgggccagcactgaaacaccgcattgtaaccaggttatctggcaaaaaaacggcgctgtgggcctttggtcttactgatgaagtgtttgccgccgcaacaaccaagctaatgaaagatcaacggcgctggagtgaaaactggatgcttggcatcgcgttcacctcttggttgtcttgggtagctggcaccgctatcggcgcgatgtttggtcatgggccgctggaaaattacccggcgattgaagcatcactctcctttatgctcccggcgctattcctcagcttcttattggcctcgttcaaacgccaatacagccttaccgttattgcttcactgaccggagccttgctgggcgtgctgctgttctctattccggtggctattttagccggtattggcggcggatgcctggcagccctgctccaacccgtccccgagaccgttatagaaaataacgagagtgataaagaggagccgaagccatgaatatggatgttgtgatcattggtttggtggtgggaacggtcaattacctgtttcgttatctgccgctgcgcctggggcctgcccgtaaacaagcaggcctgcaacgagggaaagtctccctgttgctagacagcatcgggatcgcctctatctgtgcgttgttggtggtttccagtaccccggagatagtgcataacccacagaaattaattcctacactaattggttttttagttatctgtggatgcttttataaaaccaacagtattatcttcgccaccttactgggagcactcagttacggtctgacattcaaattactgatgattttggcataa

SEQ ID NO: 35 - DNA, 1094 bp, Photorhabdus luminescens subsp. laumondii
atgcctgtttctgatacatcatcccccttaacgagtaaaaaatcttcttttactgaaggaataatagatagtttacccattgttatcggttatattcccgtcgcctttgcttttggtctcaatgccgtcaaacttggcttcaacccaatggaagccattttcttttcatgcatcatctacgccggtgcaagccagttcgtcatcacagctttactgagtgcggggacatcattatggatttctgccctaacaattatggcaatggatgtccgccatattctttatggtccatctttaaggcaccgtatcaaagataagctaacggagaaaaaaaccgttatctgggctttcggcctgacagatgaagtttttgccgccgcgactgcaaaactcattaaaaaccaccggagctggagtgaaaactggatggttgctattgcaatctgttcttggctggcctggggcgcaggtaccgcagccggtgcatttcttggtaacggttatttggaatcctatcccgctatagaagctgccatgattttcatgttaccagcactatttctcagttttcttcttgcttcttgtagaaaacaaaatagttattgtgttgcaaccgcactaaccggagcacttttagggattacatttttctcaattccagttgctattctggcaggtattgtcggtggttgtatcgcggcactgttacaaccgcaaaacaattgcaatgactcttcagaacaaaaggaaacaccatgattgatagcaagattttgctgattggactatttgttgggttagctaacttttcatttcgctatctgccactacgatttgggaaagcacgccaatctgccggcagaaaagctggaaaaacaagcattatccttgacagtattggtattgcatccatttgttctttactcatcgtatcaggtgtacctgatgtgatgagagaaagtcaaaaactacttcctaccctcataggttgtctgaccatctgtttagtcttttacaaaacaaagcaaattatactcgcaacactatttggcgcactgctttttggactaacattcaaaatatttatgaattag

SEQ ID NO: 36 - DNA, 1063 bp, Citrobacter youngae
atggatagcccgattccgcagagcggtagccgtagcgcaaccctgaccgaaggttttaaagatagcctgccgattgtgattagctatattccggttgcatttgcctttggtctgaatgcaacccgtctgggttttacaccggttgaaagcgtttttctgagctgtattatctatgccggtgcaagccagtttgttattaccaccatgctggcagcaggtagcagcctgtgggttgcagcactgaccgttatggcaatggatgttcgtcatgttctgtatggtccgagcctgcgtagccgtattgcacagcgtctgagcaaaccgaaaagcgcactgtgggcatttggcctgaccgatgaagtttttgcagcagcaaccgcaaaactggttcgtgataatcgtcgttggagcgaaaattggatgattggtattgcactgtgtagctgggcaagctgggtttttggcaccgcaattggtgcatttagcggtagcggtctgctgaaagattatccggcagttgaagcagcactgggctttatgctgcctgcactgtttatgagctttctgctggcgagctttcagcgtaaacaggcactgtgtgttaccgttgccctgaccggtgcactggcaggcgttattctgtttagcattccggcagcaattctgctgggtattgtttgtggttgtctgaccgcactgctgcagagcttttggcagggtggtccggatgagctatgaggttctgctgctgggtctgctggttggttgtgtgaattattgttttcgttatctgccgctgcgtctgggtgcaggtaatgttcgtccggcacgtcgtggtgcaaccggtatcctgctggatacaattggcattgcaagcatttgtgcactgctggtagttagcaccgcaccggaagttatgcatgatgcacgtcgttttgttccgaccctggtgggttttgttattctgggtgccagcttctataaaacccgtagcattattatcccgaccctgctgagcgcactgggttatggtctggcatggaaaatgctggtaggtctgtaa

SEQ ID NO: 37 - DNA, 1063 bp, Citrobacter freundii
atggaaagtccggttccgcagagcgaaagcagcagcgcaaccctgaccgaaggttttaaagatagcctgccgattgtgattagctatattccggttgcatttgcctttggtctgaatgcaacccgtctgggttttacaccggttgaaagcgtgttttttagctgcattatctatgccggtgcaagccagtttgttattaccaccatgctggcagcaggtagcagcctgtgggttgcagcactgaccgttatggcaatggatgttcgtcatgttctgtatggtccgagcctgcgtagccgtattgcacagcgtctgagcaaaccgaaaagcgcactgtgggcatttggcctgaccgatgaagtttttgcagcagcaaccgcaaaactggttcgtgataatcgtcgttggagcgaaaattggatgattggtattgcactgtgtagctgggcaagctgggtttttggcaccgttctgggtgcatttagcggtagcggtctgctgaaagattatccggcagttgaagcagcactgggctttatgctgcctgcactgtttatgagctttctgctggcgagctttcagcgtaaacaggcactgtgtgttaccgcagccctggcaggcgcactggctggtgttatgctgtttagcattccggcagcaattctggcaggtattgtttgtggttgtctgaccgcactgattcagagcttttggcagggtggtccggatgagctatgaagttctgctgctgggtctgctggttggttgtgtgaattattgttttcgttatctgccgctgcgtctgggtgttggtaatgttcgtccgaccaaacgtggtgcaaccggtattctgctggataccattggtattaccagcatttgtgcactgctggtagttagcaccgcaccggaagttatgcatgatgcacgtcgttttgttccgaccctggtgggttttgttatcctgggtgccagcttctataaaacccgtagcattattatcccgaccctgctgagcgcactgggttatggtctggcatggaaaatgctggttgttctgtaa